European Patent Specification EP 3 293 266 B1, published December 24, 2025. Title: IL-12 Immunotherapy for Cancer. Applicant: University Health Network Medin, Jeffrey A. Paige, Christopher J. Application PCT/CA2008/000849. The sequence listing filed with the application follows.

SEQUENCE LISTING (17 sequences)

SEQ ID NO: 1 - DNA, 12718 bp, Artificial Sequence
  pHR'.cPPT.EF.CD19delta TmpkF105YR200A.WPRE.SIN
aattacctgtggtttcatttactctaaacctgtgattcctctgaattattttcattttaaagaaattgtatttgttaaatatgtactacaaacttagtagttggaagggctaattcactcccaaagaagacaagatatccttgatctgtggatctaccacacacaaggctacttccctgattagcagaactacacaccagggccaggggtcagatatccactgacctttggatggtgctacaagctagtaccagttgagccagataaggtagaagaggccaataaaggagagaacaccagcttgttacaccctgtgagcctgcatgggatggatgacccggagagagaagtgttagagtggaggtttgacagccgcctagcatttcatcacgtggcccgagagctgcatccggagtacttcaagaactgctgatatcgagcttgctacaagggactttccgctggggactttccagggaggcgtggcctgggcgggactggggagtggcgagccctcagatcctgcatataagcagctgctttttgcctgtactgggtctctctggttagaccagatctgagcctgggagctctctggctaactagggaacccactgcttaagcctcaataaagcttgccttgagtgcttcaagtagtgtgtgcccgtctgttgtgtgactctggtaactagagatccctcagacccttttagtcagtgtggaaaatctctagcagtggcgcccgaacagggacttgaaagcgaaagggaaaccagaggagctctctcgacgcaggactcggcttgctgaagcgcgcacggcaagaggcgaggggcggcgactggtgagtacgccaaaaattttgactagcggaggctagaaggagagagatgggtgcgagagcgtcagtattaagcgggggagaattagatcgcgatgggaaaaaattcggttaaggccagggggaaagaaaaaatataaattaaaacatatagtatgggcaagcagggagctagaacgattcgcagttaatcctggcctgttagaaacatcagaaggctgtagacaaatactgggacagctacaaccatcccttcagacaggatcagaagaacttagatcattatataatacagtagcaaccctctattgtgtgcatcaaaggatagagataaaagacaccaaggaagctttagacaagatagaggaagagcaaaacaaaagtaagaccaccgcacagcaagcggccgctgatcttcagacctggaggaggagatatgagggacaattggagaagtgaattatataaatataaagtagtaaaaattgaaccattaggagtagcacccaccaaggcaaagagaagagtggtgcagagagaaaaaagagcagtgggaataggagctttgttccttgggttcttgggagcagcaggaagcactatgggcgcagcgtcaatgacgctgacggtacaggccagacaattattgtctggtatagtgcagcagcagaacaatttgctgagggctattgaggcgcaacagcatctgttgcaactcacagtctggggcatcaagcagctccaggcaagaatcctggctgtggaaagatacctaaaggatcaacagctcctggggatttggggttgctctggaaaactcatttgcaccactgctgtgccttggaatgctagttggagtaataaatctctggaacagatttggaatcacacgacctggatggagtgggacagagaaattaacaattacacaagcttaatacactccttaattgaagaatcgcaaaaccagcaagaaaagaatgaacaagaattattggaattagataaatgggcaagtttgtggaattggtttaacataacaaattggctgtggtatataaaattattcataatgatagtaggaggcttggtaggtttaagaatagtttttgctgtactttctatagtgaatagagttaggcagggatattcaccattatcgtttcagacccacctcccaaccccgaggggacccgacaggcccgaaggaatagaagaagaaggtggagagagagacagagacagatccattcgattagtgaacggatctcgacggtatcgattttaaaagaaaaggggggattggggggtacagtgcaggggaaagaatagtagacataatagcaacagacatacaaactaaagaattacaaaaacaaattacaaaaattcaaaattttatcgataagctttgcaaagatggataaagttttaaacagagaggaatctttgcagctaatggaccttctaggtcttgaaaggagtgggaattggctccggtgcccgtcagtgggcagagcgcacatcgcccacagtccccgagaagttggggggaggggtcggcaattgaaccggtgcctagagaaggtggcgcggggtaaactgggaaagtgatgtcgtgtactggctccgcctttttcccgagggtgggggagaaccgtatataagtgcagtagtcgccgtgaacgttctttttcgcaacgggtttgccgccagaacacaggtaagtgccgtgtgtggttcccgcgggcctggcctctttacgggttatggcccttgcgtgccttgaattacttccacctggctgcagtacgtgattcttgatcccgagcttcgggttggaagtgggtgggagagttcgaggccttgcgcttaaggagccccttcgcctcgtgcttgagttgaggcctggcctgggcgctggggccgccgcgtgcgaatctggtggcaccttcgcgcctgtctcgctgctttcgataagtctctagccatttaaaatttttgatgacctgctgcgacgctttttttctggcaagatagtcttgtaaatgcgggccaagatctgcacactggtatttcggtttttggggccgcgggcggcgacggggcccgtgcgtcccagcgcacatgttcggcgaggcggggcctgcgagcgcggccaccgagaatcggacgggggtagtctcaagctggccggcctgctctggtgcctggcctcgcgccgccgtgtatcgccccgccctgggcggcaaggctggcccggtcggcaccagttgcgtgagcggaaagatggccgcttcccggccctgctgcagggagctcaaaatggaggacgcggcgctcgggagagcgggcgggtgagtcacccacacaaaggaaaagggcctttccgtcctcagccgtcgcttcatgtgactccacggagtaccgggcgccgtccaggcacctcgattagttctcgagcttttggagtacgtcgtctttaggttggggggaggggttttatgcgatggagtttccccacactgagtgggtggagactgaagttaggccagcttggcacttgatgtaattctccttggaatttgccctttttgagtttggatcttggttcattctcaagcctcagacagtggttcaaagtttttttcttccatttcaggtgtcgtgaggaattcatgccacctcctcgcctcctcttcttcctcctcttcctcacccccatggaagtcaggcccgaggaacctctagtggtgaaggtggaagagggagataacgctgtgctgcagtgcctcaaggggacctcagatggccccactcagcagctgacctggtctcgggagtccccgcttaaacccttcttaaaactcagcctggggctgccaggcctgggaatccacatgaggcccctggcatcctggcttttcatcttcaacgtctctcaacagatggggggcttctacctgtgccagccggggcccccctctgagaaggcctggcagcctggctggacagtcaatgtggagggcagcggggagctgttccggtggaatgtttcggacctaggtggcctgggctgtggcctgaagaacaggtcctcagagggccccagctccccttccgggaagctcatgagccccaagctgtatgtgtgggccaaagaccgccctgagatctgggagggagagcctccgtgtgtcccaccgagggacagcctgaaccagagcctcagccaggacctcaccatggcccctggctccacactctggctgtcctgtggggtaccccctgactctgtgtccaggggccccctctcctggacccatgtgcaccccaaggggcctaagtcattgctgagcctagagctgaaggacgatcgcccggccagagatatgtgggtaatggagacgggtctgttgttgccccgggccacagctcaagacgctggaaagtattattgtcaccgtggcaacctgaccatgtcattccacctggagatcactgctcggccagtactatggcactggctgctgaggactggtggctggaaggtctcagctgtgactttggcttatctgatcttctgcctgtgttcccttgtgggcattcttcatcttgccggcggggctgcagggatggcggcccggcgcggggctctcatagtgctggagggcgtggaccgcgccgggaagagcacgcagagccgcaagctggtggaagcgctgtgcgccgcgggccaccgcgccgaactgctccggttcccggaaagatcaactgaaatcggcaaacttctgagttcctacttgcaaaagaaaagtgacgtggaggatcactcggtgcacctgcttttttctgcaaatcgctgggaacaagtgccgttaattaaggaaaagttgagccagggcgtgaccctcgtcgtggacagatacgcattttctggtgtggcctacacaggtgccaaggagaatttttccctagactggtgtaaacagccagacgtgggccttcccaaacccgacctggtcctgttcctccagttacagctggcggatgctgccaagcggggagcgtttggccatgagcgctatgagaacggggctttccaggagcgggcgctccggtgtttccaccagctcatgaaagacacgactttgaactggaagatggtggatgcttccaaaagcatcgaagctgtccatgaggacatccgcgtgctctctgaggacgccatcgccactgccacagagaagccgctgggggagctatggaagtgaggatccaagcttcaattgtggtcactcgacaatcaacctctggattacaaaatttgtgaaagattgactggtattcttaactatgttgctccttttacgctatgtggatacgctgctttaatgcctttgtatcatgctattgcttcccgtatggctttcattttctcctccttgtataaatcctggttgctgtctctttatgaggagttgtggcccgttgtcaggcaacgtggcgtggtgtgcactgtgtttgctgacgcaacccccactggttggggcattgccaccacctgtcagctcctttccgggactttcgctttccccctccctattgccacggcggaactcatcgccgcctgccttgcccgctgctggacaggggctcggctgttgggcactgacaattccgtggtgttgtcggggaagctgacgtcctttccatggctgctcgcctgtgttgccacctggattctgcgcgggacgtccttctgctacgtcccttcggccctcaatccagcggaccttccttcccgcggcctgctgccggctctgcggcctcttccgcgtcttcgccttcgccctcagacgagtcggatctccctttgggccgcctccccgcctgctcgagacctagaaaaacatggagcaatcacaagtagcaatacagcagctaccaatgctgattgtgcctggctagaagcacaagaggaggaggaggtgggttttccagtcacacctcaggtacctttaagaccaatgacttacaaggcagctgtagatcttagccactttttaaaagaaaaggggggactggaagggctaattcactcccaacgaagacaagatctgctttttgcttgtactgggtctctctggttagaccagatctgagcctgggagctctctggctaactagggaacccactgcttaagcctcaataaagcttgccttgagtgcttcaagtagtgtgtgcccgtctgttgtgtgactctggtaactagagatccctcagacccttttagtcagtgtggaaaatctctagcagtagtagttcatgtcatcttattattcagtatttataacttgcaaagaaatgaatatcagagagtgagaggccttgacattataatagatttagcaggaattgaactaggagtggagcacacaggcaaagctgcagaagtacttggaagaagccaccagagatactcacgattctgcacatacctggctaatcccagatcctaaggattacattaagtttactaacatttatataatgatttatagtttaaagtataaacttatctaatttactattctgacagatattaattaatcctcaaatatcataagagatgattactattatccccatttaacacaagaggaaactgagagggaaagatgttgaagtaattttcccacaattacagcatccgttagttacgactctatgatcttctgacacaaattccatttactcctcaccctatgactcagtcgaatatatcaaagttatggacattatgctaagtaacaaattacccttttatatagtaaatactgagtagattgagagaagaaattgtttgcaaacctgaatagcttcaagaagaagagaagtgaggataagaataacagttgtcatttaacaagttttaacaagtaacttggttagaaagggattcaaatgcataaagcaagggataaatttttctggcaacaagactatacaatataaccttaaatatgacttcaaataattgttggaacttgataaaactaattaaatattattgaagattatcaatattataaatgtaatttacttttaaaaagggaacatagaaatgtgtatcattagagtagaaaacaatccttattatcacaatttgtcaaaacaagtttgttattaacacaagtagaatactgcattcaattaagttgactgcagattttgtgttttgttaaaattagaaagagataacaacaatttgaattattgaaagtaacatgtaaatagttctacatacgttcttttgacatcttgttcaatcattgatcgaagttctttatcttggaagaatttgttccaaagactctgaaataaggaaaacaatctattatatagtctcacacctttgttttacttttagtgatttcaatttaataatgtaaatggttaaaatttattcttctctgagatcatttcacattgcagatagaaaacctgagactggggtaatttttattaaaatctaatttaatctcagaaacacatctttattctaacatcaatttttccagtttgatattatcatataaagtcagccttcctcatctgcaggttccacaacaaaaatccaaccaactgtggatcaaaaatattgggaaaaaattaaaaatagcaatacaacaataaaaaaatacaaatcagaaaaacagcacagtataacaactttatttagcatttacaatctattaggtattataagtaatctagaattaattccgtgtattctatagtgtcacctaaatcgtatgtgtatgatacataaggttatgtattaattgtagccgcgttctaacgacaatatgtacaagcctaattgtgtagcatctggcttactgaagcagaccctatcatctctctcgtaaactgccgtcagagtcggtttggttggacgaaccttctgagtttctggtaacgccgtcccgcacccggaaatggtcagcgaaccaatcagcagggtcatcgctagccagatcctctacgccggacgcatcgtggccggcatcaccggcgccacaggtgcggttgctggcgcctatatcgccgacatcaccgatggggaagatcgggctcgccacttcgggctcatgagcgcttgtttcggcgtgggtatggtggcaggccccgtggccgggggactgttgggcgccatctccttgcatgcaccattccttgcggcggcggtgctcaacggcctcaacctactactgggctgcttcctaatgcaggagtcgcataagggagagcgtcgaatggtgcactctcagtacaatctgctctgatgccgcatagttaagccagccccgacacccgccaacacccgctgacgcgccctgacgggcttgtctgctcccggcatccgcttacagacaagctgtgaccgtctccgggagctgcatgtgtcagaggttttcaccgtcatcaccgaaacgcgcgagacgaaagggcctcgtgatacgcctatttttataggttaatgtcatgataataatggtttcttagacgtcaggtggcacttttcggggaaatgtgcgcggaacccctatttgtttatttttctaaatacattcaaatatgtatccgctcatgagacaataaccctgataaatgcttcaataatattgaaaaaggaagagtatgagtattcaacatttccgtgtcgcccttattcccttttttgcggcattttgccttcctgtttttgctcacccagaaacgctggtgaaagtaaaagatgctgaagatcagttgggtgcacgagtgggttacatcgaactggatctcaacagcggtaagatccttgagagttttcgccccgaagaacgttttccaatgatgagcacttttaaagttctgctatgtggcgcggtattatcccgtattgacgccgggcaagagcaactcggtcgccgcatacactattctcagaatgacttggttgagtactcaccagtcacagaaaagcatcttacggatggcatgacagtaagagaattatgcagtgctgccataaccatgagtgataacactgcggccaacttacttctgacaacgatcggaggaccgaaggagctaaccgcttttttgcacaacatgggggatcatgtaactcgccttgatcgttgggaaccggagctgaatgaagccataccaaacgacgagcgtgacaccacgatgcctgtagcaatggcaacaacgttgcgcaaactattaactggcgaactacttactctagcttcccggcaacaattaatagactggatggaggcggataaagttgcaggaccacttctgcgctcggcccttccggctggctggtttattgctgataaatctggagccggtgagcgtgggtctcgcggtatcattgcagcactggggccagatggtaagccctcccgtatcgtagttatctacacgacggggagtcaggcaactatggatgaacgaaatagacagatcgctgagataggtgcctcactgattaagcattggtaactgtcagaccaagtttactcatatatactttagattgatttaaaacttcatttttaatttaaaaggatctaggtgaagatcctttttgataatctcatgaccaaaatcccttaacgtgagttttcgttccactgagcgtcagaccccgtagaaaagatcaaaggatcttcttgagatcctttttttctgcgcgtaatctgctgcttgcaaacaaaaaaaccaccgctaccagcggtggtttgtttgccggatcaagagctaccaactctttttccgaaggtaactggcttcagcagagcgcagataccaaatactgttcttctagtgtagccgtagttaggccaccacttcaagaactctgtagcaccgcctacatacctcgctctgctaatcctgttaccagtggctgctgccagtggcgataagtcgtgtcttaccgggttggactcaagacgatagttaccggataaggcgcagcggtcgggctgaacggggggttcgtgcacacagcccagcttggagcgaacgacctacaccgaactgagatacctacagcgtgagctatgagaaagcgccacgcttcccgaagggagaaaggcggacaggtatccggtaagcggcagggtcggaacaggagagcgcacgagggagcttccagggggaaacgcctggtatctttatagtcctgtcgggtttcgccacctctgacttgagcgtcgatttttgtgatgctcgtcaggggggcggagcctatggaaaaacgccagcaacgcggcctttttacggttcctggccttttgctggccttttgctcacatgttctttcctgcgttatcccctgattctgtggataaccgtattaccgcctttgagtgagctgataccgctcgccgcagccgaacgaccgagcgcagcgagtcagtgagcgaggaagcggaagagcgcccaatacgcaaaccgcctctccccgcgcgttggccgattcattaatgcagctgtggaatgtgtgtcagttagggtgtggaaagtccccaggctccccagcaggcagaagtatgcaaagcatgcatctcaattagtcagcaaccaggtgtggaaagtccccaggctccccagcaggcagaagtatgcaaagcatgcatctcaattagtcagcaaccatagtcccgcccctaactccgcccatcccgcccctaactccgcccagttccgcccattctccgccccatggctgactaattttttttatttatgcagaggccgaggccgcctcggcctctgagctattccagaagtagtgaggaggcttttttggaggcctaggcttttgcaaaaagcttggacacaagacaggcttgcgagatatgtttgagaataccactttatcccgcgtcagggagaggcagtgcgtaaaaagacgcggactcatgtgaaatactggtttttagtgcgccagatctctataatctcgcgcaacctattttcccctcgaacactttttaagccgtagataaacaggctgggacacttcacatgagcgaaaaatacatcgtcacctgggacatgttgcagatccatgcacgtaaactcgcaagccgactgatgccttctgaacaatggaaaggcattattgccgtaagccgtggcggtctgtaccgggtgcgttactggcgcgtgaactgggtattcgtcatgtcgataccgtttgtatttccagctacgatcacgacaaccagcgcgagcttaaagtgctgaaacgcgcagaaggcgatggcgaaggcttcatcgttattgatgacctggtggataccggtggtactgcggttgcgattcgtgaaatgtatccaaaagcgcactttgtcaccatcttcgcaaaaccggctggtcgtccgctggttgatgactatgttgttgatatcccgcaagatacctggattgaacagccgtgggatatgggcgtcgtattcgtcccgccaatctccggtcgctaatcttttcaacgcctggcactgccgggcgttgttctttttaacttcaggcgggttacaatagtttccagtaagtattctggaggctgcatccatgacacaggcaaacctgagcgaaaccctgttcaaaccccgctttaaacatcctgaaacctcgacgctagtccgccgctttaatcacggcgcacaaccgcctgtgcagtcggcccttgatggtaaaaccatccctcactggtatcgcatgattaaccgtctgatgtggatctggcgcggcattgacccacgcgaaatcctcgacgtccaggcacgtattgtgatgagcgatgccgaacgtaccgacgatgatttatacgatacggtgattggctaccgtggcggcaactggatttatgagtgggccccggatctttgtgaaggaaccttacttctgtggtgtgacataattggacaaactacctacagagatttaaagctctaaggtaaatataaaatttttaagtgtataatgtgttaaactactgattctaattgtttgtgtattttagattccaacctatggaactgatgaatgggagcagtggtggaatgcctttaatgaggaaaacctgttttgctcagaagaaatgccatctagtgatgatgaggctactgctgactctcaacattctactcctccaaaaaagaagagaaaggtagaagaccccaaggactttccttcagaattgctaagttttttgagtcatgctgtgtttagtaatagaactcttgcttgctttgctatttacaccacaaaggaaaaagctgcactgctatacaagaaaattatggaaaaatattctgtaacctttataagtaggcataacagttataatcataacatactgttttttcttactccacacaggcatagagtgtctgctattaataactatgctcaaaaattgtgtacctttagctttttaatttgtaaaggggttaataaggaatatttgatgtatagtgccttgactagagatcataatcagccataccacatttgtagaggttttacttgctttaaaaaacctcccacacctccccctgaacctgaaacataaaatgaatgcaattgttgttgttaacttgtttattgcagcttataatggttacaaataaagcaatagcatcacaaatttcacaaataaagcatttttttcactgcattctagttgtggtttgtccaaactcatcaatgtatcttatcatgtctggatcaactggataactcaagctaaccaaaatcatcccaaacttcccaccccataccctattaccactgcc

SEQ ID NO: 2 - DNA, 118 bp, Artificial Sequence
  cPPT  Seq
ttttaaaagaaaaggggggattggggggtacagtgcaggggaaagaatagtagacataatagcaacagacatacaaactaaagaattacaaaaacaaattacaaaaattcaaaatttt

SEQ ID NO: 3 - DNA, 592 bp, Artificial Sequence
  Viral
aatcaacctctggattacaaaatttgtgaaagattgactggtattcttaactatgttgctccttttacgctatgtggatacgctgctttaatgcctttgtatcatgctattgcttcccgtatggctttcattttctcctccttgtataaatcctggttgctgtctctttatgaggagttgtggcccgttgtcaggcaacgtggcgtggtgtgcactgtgtttgctgacgcaacccccactggttggggcattgccaccacctgtcagctcctttccgggactttcgctttccccctccctattgccacggcggaactcatcgccgcctgccttgcccgctgctggacaggggctcggctgttgggcactgacaattccgtggtgttgtcggggaagctgacgtcctttccatggctgctcgcctgtgttgccacctggattctgcgcgggacgtccttctgctacgtcccttcggccctcaatccagcggaccttccttcccgcggcctgctgccggctctgcggcctcttccgcgtcttcgccttcgccctcagacgagtcggatctccctttgggccgcctccccgcctg

SEQ ID NO: 4 - DNA, 5048 bp, Artificial Sequence
  pORF-hIL-12 Sequence
ggatctgcgatcgctccggtgcccgtcagtgggcagagcgcacatcgcccacagtccccgagaagttggggggaggggtcggcaattgaaccggtgcctagagaaggtggcgcggggtaaactgggaaagtgatgtcgtgtactggctccgcctttttcccgagggtgggggagaaccgtatataagtgcagtagtcgccgtgaacgttctttttcgcaacgggtttgccgccagaacacagctgaagcttcgaggggctcgcatctctccttcacgcgcccgccgccctacctgaggccgccatccacgccggttgagtcgcgttctgccgcctcccgcctgtggtgcctcctgaactgcgtccgccgtctaggtaagtttaaagctcaggtcgagaccgggcctttgtccggcgctcccttggagcctacctagactcagccggctctccacgctttgcctgaccctgcttgctcaactctacgtctttgtttcgttttctgttctgcgccgttacagatccaagctgtgaccggcgcctacgtaagtgatatctactagatttatcaaaaagagtgttgacttgtgagcgctcacaattgatacttagattcatcgagagggacacgtcgactactaaccttcttctctttcctacagctgagatcaccggcgaaggagggccaccatgggtcaccagcagttggtcatctcttggttttccctggtttttctggcatctcccctcgtggccatatgggaactgaagaaagatgtttatgtcgtagaattggattggtatccggatgcccctggagaaatggtggtcctcacctgtgacacccctgaagaagatggtatcacctggaccttggaccagagcagtgaggtcttaggctctggcaaaaccctgaccatccaagtcaaagagtttggagatgctggccagtacacctgtcacaaaggaggcgaggttctaagccattcgctcctgctgcttcacaaaaaggaagatggaatttggtccactgatattttaaaggaccagaaagaacccaaaaataagacctttctaagatgcgaggccaagaattattctggacgtttcacctgctggtggctgacgacaatcagtactgatttgacattcagtgtcaaaagcagcagaggctcttctgacccccaaggggtgacgtgcggagctgctacactctctgcagagagagtcagaggggacaacaaggagtatgagtactcagtggagtgccaggaggacagtgcctgcccagctgctgaggagagtctgcccattgaggtcatggtggatgccgttcacaagctcaagtatgaaaactacaccagcagcttcttcatcagggacatcatcaaacctgacccacccaagaacttgcagctgaagccattaaagaattctcggcaggtggaggtcagctgggagtaccctgacacctggagtactccacattcctacttctccctgacattctgcgttcaggtccagggcaagagcaagagagaaaagaaagatagagtcttcacggacaagacctcagccacggtcatctgccgcaaaaatgccagcattagcgtgcgggcccaggaccgctactatagctcatcttggagcgaatgggcatctgtgccctgcagtgttcctggagtaggggtacctggggtgggcgccagaaacctccccgtggccactccagacccaggaatgttcccatgccttcaccactcccaaaacctgctgagggccgtcagcaacatgctccagaaggccagacaaactctagaattttacccttgcacttctgaagagattgatcatgaagatatcacaaaagataaaaccagcacagtggaggcctgtttaccattggaattaaccaagaatgagagttgcctaaattccagagagacctctttcataactaatgggagttgcctggcctccagaaagacctcttttatgatggccctgtgccttagtagtatttatgaagactcgaagatgtaccaggtggagttcaagaccatgaatgcaaagcttctgatggatcctaagaggcagatctttctagatcaaaacatgctggcagttattgatgagctgatgcaggccctgaatttcaacagtgagactgtgccacaaaaatcctcccttgaagaaccggatttttataaaactaaaatcaagctctgcatacttcttcatgctttcagaattcgggcagtgactattgatagagtgatgagctatctgaatgcttcctaaaaagcgaggtccctccaaaccgttgtcatttttataaaactttgaaatgaggaaactttgataggatgtggattaagaactagggagggggaaagaaggatgggactattacatccacatgatacctctgatcaagtatttttgacatttactgtggataaattgtttttaagttttcatgaatgaattgctaagaaggggggaattcttttgctttttaccctcgactagctcgacatgataagatacattgatgagtttggacaaaccacaactagaatgcagtgaaaaaaatgctttatttgtgaaatttgtgatgctattgctttatttgtgaaatttgtgatgctattgctttatttgtaaccattataagctgcaataaacaagttaacaacaacaattgcattcattttatgtttcaggttcagggggaggtgtgggaggttttttaaagcaagtaaaacctctacaaatgtggtagatcatttaaatgttaattaagaacatgtgagcaaaaggccagcaaaaggccaggaaccgtaaaaaggccgcgttgctggcgtttttccataggctccgcccccctgacgagcatcacaaaaatcgacgctcaagtcagaggtggcgaaacccgacaggactataaagataccaggcgtttccccctggaagctccctcgtgcgctctcctgttccgaccctgccgcttaccggatacctgtccgcctttctcccttcgggaagcgtggcgctttctcaatgctcacgctgtaggtatctcagttcggtgtaggtcgttcgctccaagctgggctgtgtgcacgaaccccccgttcagcccgaccgctgcgccttatccggtaactatcgtcttgagtccaacccggtaagacacgacttatcgccactggcagcagccactggtaacaggattagcagagcgaggtatgtaggcggtgctacagagttcttgaagtggtggcctaactacggctacactagaagaacagtatttggtatctgcgctctgctgaagccagttaccttcggaaaaagagttggtagctcttgatccggcaaacaaaccaccgctggtagcggtggtttttttgtttgcaagcagcagattacgcgcagaaaaaaaggatctcaagaagatcctttgatcttttctacggggtctgacgctcagtggaacgaaaactcacgttaagggattttggtcatgagattatcaaaaaggatcttcacctagatccttttaaattaaaaatgaagttttaaatcaatctaaagtatatatgagtaaacttggtctgacagttaccaatgcttaatcagtgaggcacctatctcagcgatctgtctatttcgttcatccatagttgcctgactccccgtcgtgtagataactacgatacgggagggcttaccatctggccccagtgctgcaatgataccgcgagacccacgctcaccggctccagatttatcagcaataaaccagccagccggaagggccgagcgcagaagtggtcctgcaactttatccgcctccatccagtctattaattgttgccgggaagctagagtaagtagttcgccagttaatagtttgcgcaacgttgttgccattgctacaggcatcgtggtgtcacgctcgtcgtttggtatggcttcattcagctccggttcccaacgatcaaggcgagttacatgatcccccatgttgtgcaaaaaagcggttagctccttcggtcctccgatcgttgtcagaagtaagttggccgcagtgttatcactcatggttatggcagcactgcataattctcttactgtcatgccatccgtaagatgcttttctgtgactggtgagtactcaaccaagtcattctgagaatagtgtatgcggcgaccgagttgctcttgcccggcgtcaatacgggataataccgcgccacatagcagaactttaaaagtgctcatcattggaaaacgttcttcggggcgaaaactctcaaggatcttaccgctgttgagatccagttcgatgtaacccactcgtgcacccaactgatcttcagcatcttttactttcaccagcgtttctgggtgagcaaaaacaggaaggcaaaatgccgcaaaaaagggaataagggcgacacggaaatgttgaatactcatactcttcctttttcaatattattgaagcatttatcagggttattgtctcatgagcggatacatatttgaatgtatttagaaaaataaacaaataggggttccgcgcacatttccccgaaaagtgccacctgacgtctaagaaaccattattatcatgacattaacctataaaaataggcgtatcacgaggccctttcgtctcgcgcgtttcggtgatgacggtgaaaacctctgacacatgcagctcccggagacggtcacagcttgtctgtaagcggatgccgggagcagacaagcccgtcagggcgcgtcagcgggtgttggcgggtgtcggggctggcttaactatgcggcatcagagcagattgtactgagagtgcaccatatggatctcgagcggccgcaataaaatatctttattttcattacatctgtgtgttggttttttgtgtgaatcgtaactaacatacgctctccatcaaaacaaaacgaaacaaaacaaactagcaaaataggctgtccccagtgcaagtgcaggtgccagaacatttctctatcgaa

SEQ ID NO: 5 - DNA, 4846 bp, Artificial Sequence
  pORF-mIL-12 (p35p40) Sequence
ggatctgcgatcgctccggtgcccgtcagtgggcagagcgcacatcgcccacagtccccgagaagttggggggaggggtcggcaattgaaccggtgcctagagaaggtggcgcggggtaaactgggaaagtgatgtcgtgtactggctccgcctttttcccgagggtgggggagaaccgtatataagtgcagtagtcgccgtgaacgttctttttcgcaacgggtttgccgccagaacacagctgaagcttcgaggggctcgcatctctccttcacgcgcccgccgccctacctgaggccgccatccacgccggttgagtcgcgttctgccgcctcccgcctgtggtgcctcctgaactgcgtccgccgtctaggtaagtttaaagctcaggtcgagaccgggcctttgtccggcgctcccttggagcctacctagactcagccggctctccacgctttgcctgaccctgcttgctcaactctacgtctttgtttcgttttctgttctgcgccgttacagatccaagctgtgaccggcgcctacgtaagtgatatctactagatttatcaaaaagagtgttgacttgtgagcgctcacaattgatacttagattcatcgagagggacacgtcgactactaaccttcttctctttcctacagctgagatcaccggcgaaggagggccaccatgggtcaatcacgctacctcctctttttggccacccttgccctcctaaaccacctcagtttggccagggtcattccagtctctggacctgccaggtgtcttagccagtcccgaaacctgctgaagaccacagatgacatggtgaagacggccagagaaaagctgaaacattattcctgcactgctgaagacatcgatcatgaagacatcacacgggaccaaaccagcacattgaagacctgtttaccactggaactacacaagaacgagagttgcctggctactagagagacttcttccacaacaagagggagctgcctgcccccacagaagacgtctttgatgatgaccctgtgccttggtagcatctatgaggacttgaagatgtaccagacagagttccaggccatcaacgcagcacttcagaatcacaaccatcagcagatcattctagacaagggcatgctggtggccatcgatgagctgatgcagtctctgaatcataatggcgagactctgcgccagaaacctcctgtgggagaagcagacccttacagagtgaaaatgaagctctgcatcctgcttcacgccttcagcacccgcgtcgtgaccatcaacagggtgatgggctatctgagctccgccgttcctggagtaggggtacctggagtgggcggatctatgtgggagctggagaaagacgtttatgttgtagaggtggactggactcccgatgcccctggagaaacagtgaacctcacctgtgacacgcctgaagaagatgacatcacctggacctcagaccagagacatggagtcataggctctggaaagaccctgaccatcactgtcaaagagtttctagatgctggccagtacacctgccacaaaggaggcgagactctgagccactcacatctgctgctccacaagaaggaaaatggaatttggtccactgaaattttaaaaaatttcaaaaacaagactttcctgaagtgtgaagcaccaaattactccggacggttcacgtgctcatggctggtgcaaagaaacatggacttgaagttcaacatcaagagcagtagcagtccccccgactctcgggcagtgacatgtggaatggcgtctctgtctgcagagaaggtcacactggaccaaagggactatgagaagtattcagtgtcctgccaggaggatgtcacctgcccaactgccgaggagaccctgcccattgaactggcgttggaagcacggcagcagaataaatatgagaactacagcaccagcttcttcatcagggacatcatcaaaccagacccgcccaagaacttgcagatgaagcctttgaagaactcacaggtggaggtcagctgggagtaccctgactcctggagcactccccattcctacttctccctcaagttctttgttcgaatccagcgcaagaaagaaaagatgaaggagacagaggaggggtgtaaccagaaaggtgcgttcctcgtagagaagacatctaccgaagtccaatgcaaaggcgggaatgtctgcgtgcaagctcaggatcgctattacaattcctcatgcagcaagtgggcatgtgttccctgcagggtccgatcctaggatgcaacggatgctagctcgacatgataagatacattgatgagtttggacaaaccacaactagaatgcagtgaaaaaaatgctttatttgtgaaatttgtgatgctattgctttatttgtgaaatttgtgatgctattgctttatttgtaaccattataagctgcaataaacaagttaacaacaacaattgcattcattttatgtttcaggttcagggggaggtgtgggaggttttttaaagcaagtaaaacctctacaaatgtggtagatcatttaaatgttaattaagaacatgtgagcaaaaggccagcaaaaggccaggaaccgtaaaaaggccgcgttgctggcgtttttccataggctccgcccccctgacgagcatcacaaaaatcgacgctcaagtcagaggtggcgaaacccgacaggactataaagataccaggcgtttccccctggaagctccctcgtgcgctctcctgttccgaccctgccgcttaccggatacctgtccgcctttctcccttcgggaagcgtggcgctttctcaatgctcacgctgtaggtatctcagttcggtgtaggtcgttcgctccaagctgggctgtgtgcacgaaccccccgttcagcccgaccgctgcgccttatccggtaactatcgtcttgagtccaacccggtaagacacgacttatcgccactggcagcagccactggtaacaggattagcagagcgaggtatgtaggcggtgctacagagttcttgaagtggtggcctaactacggctacactagaagaacagtatttggtatctgcgctctgctgaagccagttaccttcggaaaaagagttggtagctcttgatccggcaaacaaaccaccgctggtagcggtggtttttttgtttgcaagcagcagattacgcgcagaaaaaaaggatctcaagaagatcctttgatcttttctacggggtctgacgctcagtggaacgaaaactcacgttaagggattttggtcatgagattatcaaaaaggatcttcacctagatccttttaaattaaaaatgaagttttaaatcaatctaaagtatatatgagtaaacttggtctgacagttaccaatgcttaatcagtgaggcacctatctcagcgatctgtctatttcgttcatccatagttgcctgactccccgtcgtgtagataactacgatacgggagggcttaccatctggccccagtgctgcaatgataccgcgagacccacgctcaccggctccagatttatcagcaataaaccagccagccggaagggccgagcgcagaagtggtcctgcaactttatccgcctccatccagtctattaattgttgccgggaagctagagtaagtagttcgccagttaatagtttgcgcaacgttgttgccattgctacaggcatcgtggtgtcacgctcgtcgtttggtatggcttcattcagctccggttcccaacgatcaaggcgagttacatgatcccccatgttgtgcaaaaaagcggttagctccttcggtcctccgatcgttgtcagaagtaagttggccgcagtgttatcactcatggttatggcagcactgcataattctcttactgtcatgccatccgtaagatgcttttctgtgactggtgagtactcaaccaagtcattctgagaatagtgtatgcggcgaccgagttgctcttgcccggcgtcaatacgggataataccgcgccacatagcagaactttaaaagtgctcatcattggaaaacgttcttcggggcgaaaactctcaaggatcttaccgctgttgagatccagttcgatgtaacccactcgtgcacccaactgatcttcagcatcttttactttcaccagcgtttctgggtgagcaaaaacaggaaggcaaaatgccgcaaaaaagggaataagggcgacacggaaatgttgaatactcatactcttcctttttcaatattattgaagcatttatcagggttattgtctcatgagcggatacatatttgaatgtatttagaaaaataaacaaataggggttccgcgcacatttccccgaaaagtgccacctgacgtctaagaaaccattattatcatgacattaacctataaaaataggcgtatcacgaggccctttcgtctcgcgcgtttcggtgatgacggtgaaaacctctgacacatgcagctcccggagacggtcacagcttgtctgtaagcggatgccgggagcagacaagcccgtcagggcgcgtcagcgggtgttggcgggtgtcggggctggcttaactatgcggcatcagagcagattgtactgagagtgcaccatatggatctcgagcggccgcaataaaatatctttattttcattacatctgtgtgttggttttttgtgtgaatcgtaactaacatacgctctccatcaaaacaaaacgaaacaaaacaaactagcaaaataggctgtccccagtgcaagtgcaggtgccagaacatttctctatcgaa

SEQ ID NO: 6 - DNA, 639 bp, Homo sapiens tmpk wt
atggcggcccggcgcggggctctcatagtgctggagggcgtggaccgcgccgggaagagcacgcagagccgcaagctggtggaagcgctgtgcgccgcgggccaccgcgccgaactgctccggttcccggaaagatcaactgaaatcggcaaacttctgagttcctacttgcaaaagaaaagtgacgtggaggatcactcggtgcacctgcttttttctgcaaatcgctgggaacaagtgccgttaattaaggaaaagttgagccagggcgtgaccctcgtcgtggacagatacgcattttctggtgtggccttcaccggtgccaaggagaatttttccctagattggtgtaaacagccagacgtgggccttcccaaacccgacctggtcctgttcctccagttacagctggcggatgctgccaagcggggagcgtttggccatgagcgctatgagaacggggctttccaggagcgggcgctccggtgtttccaccagctcatgaaagacacgactttgaactggaagatggtggatgcttccaaaagcatcgaagctgtccatgaggacatccgcgtgctctctgaggacgccatccgcactgccacagagaagccgctgggggagctatggaagtga

SEQ ID NO: 7 - protein, 212 aa, Homo sapiens tmpk wt
MAARRGALIVLEGVDRAGKSTQSRKLVEALCAAGHRAELLRFPERSTEIGKLLSSYLQKKSDVEDHSVHLLFSANRWEQVPLIKEKLSQGVTLVVDRYAFSGVAFTGAKENFSLDWCKQPDVGLPKPDLVLFLQLQLADAAKRGAFGHERYENGAFQERALRCFHQLMKDTTLNWKMVDASKSIEAVHEDIRVLSEDAIRTATEKPLGELWK

SEQ ID NO: 8 - DNA, 639 bp, Homo sapiens tmpk wt; identical to SEQ ID NO: 6

SEQ ID NO: 9 - protein, 212 aa, Homo sapiens tmpk wt; identical to SEQ ID NO: 7

SEQ ID NO: 10 - DNA, 636 bp, Homo sapiens tmpk wt
atggcggcccggcgcggggctctcatagtgctggagggcgtggaccgcgccgggaagagcacgcagagccgcaagctggtggaagcgctgtcgcgcgggccaccgcccgaactgctccggttcccggaaagatcaactgaaatcggcaaacttctgagttcctacttgcaaaagaaaagtgacgtggaggatcactcggtgcacctgcttttttctgcaaatcgctgggaacaagtgccgttaattaaggaaaagttgagccagggcgtgaccctcgtcgtggacagatacgcattttctggtgtggccttcaccggtgccaaggagaatttttccctagactggtgtaaacagccagacgtgggccttcccaaacccgacctggtcctgttcctccagttacagctggcggatgctgccaagcggggagcgtttggccatgagcgctatgagaacggggctttccaggagcgggcgctccggtgtttccaccagctcatgaaagacacgactttgaactggaagatggtggatgcttccaaaagactcgaagctgtccatgaggaactccgcgtgctctctgaggacgccatccgcactgccacagagaagccgctgggggagctatggaagtga

SEQ ID NO: 11 - protein, 211 aa, Homo sapiens tmpk wt
MAARRGALIVLEGVDRAGKSTQSRKLVEALSRGPPPELLRFPERSTEIGKLLSSYLQKKSDVEDHSVHLLFSANRWEQVPLIKEKLSQGVTLVVDRYAFSGVAFTGAKENFSLDWCKQPDVGLPKPDLVLFLQLQLADAAKRGAFGHERYENGAFQERALRCFHQLMKDTTLNWKMVDASKRLEAVHEELRVLSEDAIRTATEKPLGELWK

SEQ ID NO: 12 - DNA, 639 bp, Homo sapiens tmpk wt (no stop codon)
atggcggcccggcgcggggctctcatagtgctggagggcgtggaccgcgccgggaagagcacgcagagccgcaagctggtggaagcgctgtgcgccgcgggccaccgcgccgaactgctccggttcccggaaagatcaactgaaatcggcaaacttctgagttcctacttgcaaaagaaaagtgacgtggaggatcactcggtgcacctgcttttttctgcaaatcgctgggaacaagtgccgttaattaaggaaaagttgagccagggcgtgaccctcgtcgtggacagatacgcattttctggtgtggccttcaccggtgccaaggagaatttttccctagattggtgtaaacagccagacgtgggccttcccaaacccgacctggtcctgttcctccagttacagctggcggatgctgccaagcggggagcgtttggccatgagcgctatgagaacggggctttccaggagcgggcgctccggtgtttccaccagctcatgaaagacacgactttgaactggaagatggtggatgcttccaaaagcatcgaagctgtccatgaggacatccgcgtgctctctgaggacgccatccgcactgccacagagaagccgctgggggagctatggaaggac

SEQ ID NO: 13 - protein, 213 aa, Homo sapiens tmpk wt putative sequence
MAARRGALIVLEGVDRAGKSTQSRKLVEALCAAGHRAELLRFPERSTEIGKLLSSYLQKKSDVEDHSVHLLFSANRWEQVPLIKEKLSQGVTLVVDRYAFSGVAFTGAKENFSLDWCKQPDVGLPKPDLVLFLQLQLADAAKRGAFGHERYENGAFQERALRCFHQLMKDTTLNWKMVDASKSIEAVHEDIRVLSEDAIRTATEKPLGELWKD

SEQ ID NO: 14 - DNA, 639 bp, Mus musculus tmpk wt
atggcgtcgcgtcggggagcgctcatcgtgctggagggtgtggaccgtgctggcaagaccacgcagggcctcaagctggtgaccgcgctgtgcgcctcgggccacagagcggagctgctgcgtttccccgaaagatcaacggaaatcggcaagcttctgaattcctacttggaaaagaaaacggaactagaggatcactccgtgcacctgctcttctctgcaaaccgctgggaacaagtaccattaattaaggcgaagttgaaccagggtgtgacccttgttttggacagatacgccttttctggggttgccttcactggtgccaaagagaatttttccctggattggtgtaaacaaccggacgtgggccttcccaaacctgacctgatcctgttccttcagttacaattgctggacgctgctgcacggggagagtttggccttgagcgatatgagaccgggactttccaaaagcaggttctgttgtgtttccagcagctcatggaagagaaaaacctcaactggaaggtggttgatgcttccaaaagcattgaggaagtccataaagaaatccgtgcacactctgaggacgccatccgaaacgctgcacagaggccactgggggagctatggaaataa

SEQ ID NO: 15 - protein, 212 aa, Mus musculus tmpk wt
MASRRGALIVLEGVDRAGKTTQGLKLVTALCASGHRAELLRFPERSTEIGKLLNSYLEKKTELEDHSVHLLFSANRWEQVPLIKAKLNQGVTLVLDRYAFSGVAFTGAKENFSLDWCKQPDVGLPKPDLILFLQLQLLDAAARGEFGLERYETGTFQKQVLLCFQQLMEEKNLNWKVVDASKSIEEVHKEIRAHSEDAIRNAAQRPLGELWK

SEQ ID NO: 16 - protein, 212 aa, Homo sapiens tmpk F1O5Y mutant
MAARRGALIVLEGVDRAGKSTQSRKLVEALCAAGHRAELLRFPERSTEIGKLLSSYLQKKSDVEDHSVHLLFSANRWEQVPLIKEKLSQGVTLVVDRYAFSGVAYTGAKENFSLDWCKQPDVGLPKPDLVLFLQLQLADAAKRGAFGHERYENGAFQERALRCFHQLMKDTTLNWKMVDASKSIEAVHEDIRVLSEDAIRTATEKPLGELWK

SEQ ID NO: 17 - protein, 214 aa, Homo sapiens tmpk R16GLL mutant
MAARRGALIVLEGVDGAGKSTQSRKLVEALCAAGHRAELLRFPERSTEIGKLLSSYLQKKSDVEDHSVHLLFSANRWEQVPLIKEKLSQGVTLVVDRYAFSGVAFTGAKENFSLDWCKQPDVGLPKPDLVLFLQLTPEVGLKRARARGQLDRYENGAFQERALRCFHQLMKDTTLNWKMVDASKSIEAVHEDIRVLSEDAIATATEKPLGELWK